European Patent Application EP 4 410 982 A1, published August 7, 2024. Title: PRODUCTION METHOD OF POLYPEPTIDE, TAG, EXPRESSION VECTOR, EVALUATION METHOD OF POLYPEPTIDE, PRODUCTION METHOD OF NUCLEIC ACID DISPLAY LIBRARY, AND SCREENING METHOD. Applicant: 富士フイルム株式会社. The sequence listing filed with the application follows.

SEQUENCE LISTING (139 sequences)

SEQ ID NO: 1-3 - skipped (3 entries)

SEQ ID NO: 4 - protein, 10 aa, synthetic construct
  REGION 1..10: note = VKKX Tag
  SITE 7..10: note = UNSURE
VKKTKTXXXX

SEQ ID NO: 5 - protein, 39 aa, synthetic construct
  REGION 1..39: note = Fusion protein
  SITE 11: note = Chloroacetyl lysine
ACIPRGDSFAXAGGSEQKLISEEDLGGSVSGWRLFKKIS

SEQ ID NO: 6 - DNA, 120 bp, synthetic construct
  misc_feature 1..120: note = Code sequence of fusion protein
  misc_feature 31..33: note = tag is a triplet to be translated
  source 1..120: mol_type = other DNA
gcgtgcatcccgcgcggcgattcttttgcataggcaggcggttctgaacagaaactgatcagcgaagaagatctgggtggctctgtaagtggatggcgattattcaagaagattagctaa

SEQ ID NO: 7 - protein, 4 aa, synthetic construct
  REGION 1..4: note = VKKX Tag
VKKI

SEQ ID NO: 8 - protein, 4 aa, synthetic construct
  REGION 1..4: note = VKKX Tag
VKKK

SEQ ID NO: 9 - protein, 4 aa, synthetic construct
  REGION 1..4: note = VKKX Tag
VKKT

SEQ ID NO: 10 - protein, 4 aa, synthetic construct
  REGION 1..4: note = VKKX Tag
VKKR

SEQ ID NO: 11 - protein, 4 aa, synthetic construct
  REGION 1..4: note = VKKX Tag
VKKS

SEQ ID NO: 12 - protein, 4 aa, synthetic construct
  REGION 1..4: note = VKKX Tag
VKKH

SEQ ID NO: 13 - protein, 4 aa, synthetic construct
  REGION 1..4: note = VKKX Tag
VKKM

SEQ ID NO: 14 - protein, 4 aa, synthetic construct
  REGION 1..4: note = VKKX Tag
VKKP

SEQ ID NO: 15 - protein, 4 aa, synthetic construct
  REGION 1..4: note = VKKX Tag
VKKG

SEQ ID NO: 16 - protein, 4 aa, synthetic construct
  REGION 1..4: note = VKKX Tag
VKKL

SEQ ID NO: 17 - protein, 4 aa, synthetic construct
  REGION 1..4: note = VKKX Tag
VKKV

SEQ ID NO: 18 - protein, 4 aa, synthetic construct
  REGION 1..4: note = VKKX Tag
VKKE

SEQ ID NO: 19 - protein, 4 aa, synthetic construct
  REGION 1..4: note = VKKX Tag
VKKA

SEQ ID NO: 20 - protein, 4 aa, synthetic construct
  REGION 1..4: note = VKKX Tag
VKKD

SEQ ID NO: 21 - protein, 4 aa, synthetic construct
  REGION 1..4: note = VKKX Tag
VKKC

SEQ ID NO: 22 - protein, 4 aa, synthetic construct
  REGION 1..4: note = VKKX Tag
VKKN

SEQ ID NO: 23 - protein, 4 aa, synthetic construct
  REGION 1..4: note = VKKX Tag
VKKY

SEQ ID NO: 24 - protein, 4 aa, synthetic construct
  REGION 1..4: note = VKKX Tag
VKKQ

SEQ ID NO: 25 - protein, 4 aa, synthetic construct
  REGION 1..4: note = VKKX Tag
VKKW

SEQ ID NO: 26 - protein, 4 aa, synthetic construct
  REGION 1..4: note = VKKX Tag
VKKF

SEQ ID NO: 27 - protein, 6 aa, synthetic construct
  REGION 1..6: note = VKKX Tag
VKKTKT

SEQ ID NO: 28 - protein, 7 aa, synthetic construct
  REGION 1..7: note = VKKX Tag
VKKTKTT

SEQ ID NO: 29 - protein, 7 aa, synthetic construct
  REGION 1..7: note = VKKX Tag
VKKTKTD

SEQ ID NO: 30 - protein, 8 aa, synthetic construct
  REGION 1..8: note = VKKX Tag
VKKTKTKK

SEQ ID NO: 31 - protein, 8 aa, synthetic construct
  REGION 1..8: note = VKKX Tag
VKKTKTKT

SEQ ID NO: 32 - protein, 8 aa, synthetic construct
  REGION 1..8: note = VKKX Tag
VKKTKTKD

SEQ ID NO: 33 - protein, 8 aa, synthetic construct
  REGION 1..8: note = VKKX Tag
VKKTKTTK

SEQ ID NO: 34 - protein, 8 aa, synthetic construct
  REGION 1..8: note = VKKX Tag
VKKTKTTT

SEQ ID NO: 35 - protein, 8 aa, synthetic construct
  REGION 1..8: note = VKKX Tag
VKKTKTDD

SEQ ID NO: 36 - protein, 9 aa, synthetic construct
  REGION 1..9: note = VKKX Tag
VKKTKTKKT

SEQ ID NO: 37 - protein, 9 aa, synthetic construct
  REGION 1..9: note = VKKX Tag
VKKTKTKKD

SEQ ID NO: 38 - protein, 9 aa, synthetic construct
  REGION 1..9: note = VKKX Tag
VKKTKTKTK

SEQ ID NO: 39 - protein, 9 aa, synthetic construct
  REGION 1..9: note = VKKX Tag
VKKTKTKTT

SEQ ID NO: 40 - protein, 9 aa, synthetic construct
  REGION 1..9: note = VKKX Tag
VKKTKTKDK

SEQ ID NO: 41 - protein, 9 aa, synthetic construct
  REGION 1..9: note = VKKX Tag
VKKTKTKDT

SEQ ID NO: 42 - protein, 9 aa, synthetic construct
  REGION 1..9: note = VKKX Tag
VKKTKTKDD

SEQ ID NO: 43 - protein, 9 aa, synthetic construct
  REGION 1..9: note = VKKX Tag
VKKTKTTKK

SEQ ID NO: 44 - protein, 9 aa, synthetic construct
  REGION 1..9: note = VKKX Tag
VKKTKTTKT

SEQ ID NO: 45 - protein, 9 aa, synthetic construct
  REGION 1..9: note = VKKX Tag
VKKTKTTKD

SEQ ID NO: 46 - protein, 10 aa, synthetic construct
  REGION 1..10: note = VKKX Tag
VKKTKTKKTK

SEQ ID NO: 47 - protein, 10 aa, synthetic construct
  REGION 1..10: note = VKKX Tag
VKKTKTKKDK

SEQ ID NO: 48 - protein, 10 aa, synthetic construct
  REGION 1..10: note = VKKX Tag
VKKTKTKTKK

SEQ ID NO: 49 - protein, 10 aa, synthetic construct
  REGION 1..10: note = VKKX Tag
VKKTKTKTTK

SEQ ID NO: 50 - protein, 10 aa, synthetic construct
  REGION 1..10: note = VKKX Tag
VKKTKTKDKK

SEQ ID NO: 51 - protein, 10 aa, synthetic construct
  REGION 1..10: note = VKKX Tag
VKKTKTTTKK

SEQ ID NO: 52 - protein, 11 aa, synthetic construct
  REGION 1..11: note = VKKX Tag
VKKTKTKTDTT

SEQ ID NO: 53 - DNA, 12 bp, synthetic construct
  misc_feature 1..12: note = Code sequence of VKKX Tag
  source 1..12: mol_type = other DNA
gttaaaaaaata

SEQ ID NO: 54 - DNA, 12 bp, synthetic construct
  misc_feature 1..12: note = Code sequence of VKKX Tag
  source 1..12: mol_type = other DNA
gttaaaaaaaaa

SEQ ID NO: 55 - DNA, 12 bp, synthetic construct
  misc_feature 1..12: note = Code sequence of VKKX Tag
  source 1..12: mol_type = other DNA
gttaaaaaaaca

SEQ ID NO: 56 - DNA, 12 bp, synthetic construct
  misc_feature 1..12: note = Code sequence of VKKX Tag
  source 1..12: mol_type = other DNA
gttaaaaaacgg

SEQ ID NO: 57 - DNA, 12 bp, synthetic construct
  misc_feature 1..12: note = Code sequence of VKKX Tag
  source 1..12: mol_type = other DNA
gttaaaaaatca

SEQ ID NO: 58 - DNA, 12 bp, synthetic construct
  misc_feature 1..12: note = Code sequence of VKKX Tag
  source 1..12: mol_type = other DNA
gttaaaaaacat

SEQ ID NO: 59 - DNA, 12 bp, synthetic construct
  misc_feature 1..12: note = Code sequence of VKKX Tag
  source 1..12: mol_type = other DNA
gttaaaaaaatg

SEQ ID NO: 60 - DNA, 12 bp, synthetic construct
  misc_feature 1..12: note = Code sequence of VKKX Tag
  source 1..12: mol_type = other DNA
gttaaaaaacct

SEQ ID NO: 61 - DNA, 12 bp, synthetic construct
  misc_feature 1..12: note = Code sequence of VKKX Tag
  source 1..12: mol_type = other DNA
gttaaaaaaggc

SEQ ID NO: 62 - DNA, 12 bp, synthetic construct
  misc_feature 1..12: note = Code sequence of VKKX Tag
  source 1..12: mol_type = other DNA
gttaaaaaacta

SEQ ID NO: 63 - DNA, 12 bp, synthetic construct
  misc_feature 1..12: note = Code sequence of VKKX Tag
  source 1..12: mol_type = other DNA
gttaaaaaagtt

SEQ ID NO: 64 - DNA, 12 bp, synthetic construct
  misc_feature 1..12: note = Code sequence of VKKX Tag
  source 1..12: mol_type = other DNA
gttaaaaaagaa

SEQ ID NO: 65 - DNA, 12 bp, synthetic construct
  misc_feature 1..12: note = Code sequence of VKKX Tag
  source 1..12: mol_type = other DNA
gttaaaaaagca

SEQ ID NO: 66 - DNA, 12 bp, synthetic construct
  misc_feature 1..12: note = Code sequence of VKKX Tag
  source 1..12: mol_type = other DNA
gttaaaaaagat

SEQ ID NO: 67 - DNA, 12 bp, synthetic construct
  misc_feature 1..12: note = Code sequence of VKKX Tag
  source 1..12: mol_type = other DNA
gttaaaaaatgt

SEQ ID NO: 68 - DNA, 12 bp, synthetic construct
  misc_feature 1..12: note = Code sequence of VKKX Tag
  source 1..12: mol_type = other DNA
gttaaaaaaaat

SEQ ID NO: 69 - DNA, 12 bp, synthetic construct
  misc_feature 1..12: note = Code sequence of VKKX Tag
  source 1..12: mol_type = other DNA
gttaaaaaatat

SEQ ID NO: 70 - DNA, 12 bp, synthetic construct
  misc_feature 1..12: note = Code sequence of VKKX Tag
  source 1..12: mol_type = other DNA
gttaaaaaacaa

SEQ ID NO: 71 - DNA, 12 bp, synthetic construct
  misc_feature 1..12: note = Code sequence of VKKX Tag
  source 1..12: mol_type = other DNA
gttaaaaaatgg

SEQ ID NO: 72 - DNA, 12 bp, synthetic construct
  misc_feature 1..12: note = Code sequence of VKKX Tag
  source 1..12: mol_type = other DNA
gttaaaaaattt

SEQ ID NO: 73 - DNA, 18 bp, synthetic construct
  misc_feature 1..18: note = Code sequence of VKKX Tag
  source 1..18: mol_type = other DNA
gttaaaaaaacaaaaaca

SEQ ID NO: 74 - DNA, 21 bp, synthetic construct
  misc_feature 1..21: note = Code sequence of VKKX Tag
  source 1..21: mol_type = other DNA
gttaaaaaaacaaaaacaaca

SEQ ID NO: 75 - DNA, 21 bp, synthetic construct
  misc_feature 1..21: note = Code sequence of VKKX Tag
  source 1..21: mol_type = other DNA
gttaaaaaaacaaaaacagat

SEQ ID NO: 76 - DNA, 24 bp, synthetic construct
  misc_feature 1..24: note = Code sequence of VKKX Tag
  source 1..24: mol_type = other DNA
gttaaaaaaacaaaaacaaaaaaa

SEQ ID NO: 77 - DNA, 24 bp, synthetic construct
  misc_feature 1..24: note = Code sequence of VKKX Tag
  source 1..24: mol_type = other DNA
gttaaaaaaacaaaaacaaaaaca

SEQ ID NO: 78 - DNA, 24 bp, synthetic construct
  misc_feature 1..24: note = Code sequence of VKKX Tag
  source 1..24: mol_type = other DNA
gttaaaaaaacaaaaacaaaagat

SEQ ID NO: 79 - DNA, 24 bp, synthetic construct
  misc_feature 1..24: note = Code sequence of VKKX Tag
  source 1..24: mol_type = other DNA
gttaaaaaaacaaaaacaacaaaa

SEQ ID NO: 80 - DNA, 24 bp, synthetic construct
  misc_feature 1..24: note = Code sequence of VKKX Tag
  source 1..24: mol_type = other DNA
gttaaaaaaacaaaaacaacaaca

SEQ ID NO: 81 - DNA, 24 bp, synthetic construct
  misc_feature 1..24: note = Code sequence of VKKX Tag
  source 1..24: mol_type = other DNA
gttaaaaaaacaaaaacagatgat

SEQ ID NO: 82 - DNA, 27 bp, synthetic construct
  misc_feature 1..27: note = Code sequence of VKKX Tage
  source 1..27: mol_type = other DNA
gttaaaaaaacaaaaacaaaaaaaaca

SEQ ID NO: 83 - DNA, 27 bp, synthetic construct
  misc_feature 1..27: note = Code sequence of VKKX Tag
  source 1..27: mol_type = other DNA
gttaaaaaaacaaaaacaaaaaaagat

SEQ ID NO: 84 - DNA, 27 bp, synthetic construct
  misc_feature 1..27: note = Code sequence of VKKX Tag
  source 1..27: mol_type = other DNA
gttaaaaaaacaaaaacaaaaacaaaa

SEQ ID NO: 85 - DNA, 27 bp, synthetic construct
  misc_feature 1..27: note = Code sequence of VKKX Tag
  source 1..27: mol_type = other DNA
gttaaaaaaacaaaaacaaaaacaaca

SEQ ID NO: 86 - DNA, 27 bp, synthetic construct
  misc_feature 1..27: note = Code sequence of VKKX Tag
  source 1..27: mol_type = other DNA
gttaaaaaaacaaaaacaaaagataaa

SEQ ID NO: 87 - DNA, 27 bp, synthetic construct
  misc_feature 1..27: note = Code sequence of VKKX Tag
  source 1..27: mol_type = other DNA
gttaaaaaaacaaaaacaaaagataca

SEQ ID NO: 88 - DNA, 27 bp, synthetic construct
  misc_feature 1..27: note = Code sequence of VKKX Tag
  source 1..27: mol_type = other DNA
gttaaaaaaacaaaaacaaaagatgat

SEQ ID NO: 89 - DNA, 27 bp, synthetic construct
  misc_feature 1..27: note = Code sequence of VKKX Tag
  source 1..27: mol_type = other DNA
gttaaaaaaacaaaaacaacaaaaaaa

SEQ ID NO: 90 - DNA, 27 bp, synthetic construct
  misc_feature 1..27: note = Code sequence of VKKX Tag
  source 1..27: mol_type = other DNA
gttaaaaaaacaaaaacaacaaaaaca

SEQ ID NO: 91 - DNA, 27 bp, synthetic construct
  misc_feature 1..27: note = Code sequence of VKKX Tag
  source 1..27: mol_type = other DNA
gttaaaaaaacaaaaacaacaaaagat

SEQ ID NO: 92 - DNA, 30 bp, synthetic construct
  misc_feature 1..30: note = Code sequence of VKKX Tag
  source 1..30: mol_type = other DNA
gttaaaaaaacaaaaacaaaaaaaacaaaa

SEQ ID NO: 93 - DNA, 30 bp, synthetic construct
  misc_feature 1..30: note = Code sequence of VKKX Tag
  source 1..30: mol_type = other DNA
gttaaaaaaacaaaaacaaaaaaagataaa

SEQ ID NO: 94 - DNA, 30 bp, synthetic construct
  misc_feature 1..30: note = Code sequence of VKKX Tag
  source 1..30: mol_type = other DNA
gttaaaaaaacaaaaacaaaaacaaaaaaa

SEQ ID NO: 95 - DNA, 30 bp, synthetic construct
  misc_feature 1..30: note = Code sequence of VKKX Tag
  source 1..30: mol_type = other DNA
gttaaaaaaacaaaaacaaaaacaacaaaa

SEQ ID NO: 96 - DNA, 30 bp, synthetic construct
  misc_feature 1..30: note = Code sequence of VKKX Tag
  source 1..30: mol_type = other DNA
gttaaaaaaacaaaaacaaaagataaaaaa

SEQ ID NO: 97 - DNA, 30 bp, synthetic construct
  misc_feature 1..30: note = Code sequence of VKKX Tag
  source 1..30: mol_type = other DNA
gttaaaaaaacaaaaacaacaacaaaaaaa

SEQ ID NO: 98 - DNA, 33 bp, synthetic construct
  misc_feature 1..33: note = Code sequence of VKKX Tag
  source 1..33: mol_type = other DNA
gttaaaaaaacaaaaacaaaaacagatacaaca

SEQ ID NO: 99 - DNA, 85 bp, synthetic construct
  misc_feature 1..85: note = Synthetic oligonucleotide
  source 1..85: mol_type = other DNA
gaaattaatacgactcactatagggagaccacaacggtttccctctagaaataattttgtttaactttaagaaggagatatacca

SEQ ID NO: 100 - DNA, 51 bp, synthetic construct
  misc_feature 1..51: note = Synthetic oligonucleotide
  source 1..51: mol_type = other DNA
cgcgcgggatgcacgctgtttttgtttttttaaccattggtatatctcctt

SEQ ID NO: 101 - DNA, 30 bp, synthetic construct
  misc_feature 1..30: note = 1st forward primer
  source 1..30: mol_type = other DNA
gaaattaatacgactcactatagggagacc

SEQ ID NO: 102 - DNA, 36 bp, synthetic construct
  misc_feature 1..36: note = 1st reverse primer
  source 1..36: mol_type = other DNA
cctgcctatgcaaaagaatcgccgcgcgggatgcac

SEQ ID NO: 103 - DNA, 74 bp, synthetic construct
  misc_feature 1..74: note = Synthetic oligonucleotide
  source 1..74: mol_type = other DNA
ggattagttattcattacagatcttcttcgctgatcagtttctgttcagaaccgcctgcctatgcaaaagaatc

SEQ ID NO: 104 - DNA, 23 bp, synthetic construct
  misc_feature 1..23: note = 2nd forward primer
  source 1..23: mol_type = other DNA
gaaattaatacgactcactatag

SEQ ID NO: 105 - DNA, 23 bp, synthetic construct
  misc_feature 1..23: note = 2nd reverse primer
  source 1..23: mol_type = other DNA
ggattagttattcattacagatc

SEQ ID NO: 106 - DNA, 240 bp, synthetic construct
  misc_feature 1..240: note = PCR product
  source 1..240: mol_type = other DNA
gaaattaatacgactcactatagggagaccacaacggtttccctctagaaataattttgtttaactttaagaaggagatataccaatggttaaaaaaacaaaaacagcgtgcatcccgcgcggcgattcttttgcataggcaggcggttctgaacagaaactgatcagcgaagaagatctgggtggctctgtaagtggatggcgattattcaagaagattagctaatgaataactaatcc

SEQ ID NO: 107 - protein, 4 aa, synthetic construct
  REGION 1..4: note = SKIK Tag
SKIK

SEQ ID NO: 108 - DNA, 12 bp, synthetic construct
  misc_feature 1..12: note = Code sequence of SKIK Tag
  source 1..12: mol_type = other DNA
agtaaaattaaa

SEQ ID NO: 109 - DNA, 12 bp, synthetic construct
  misc_feature 1..12: note = Code sequence of SKIK Tag
  source 1..12: mol_type = other DNA
agtaagattaag

SEQ ID NO: 110 - DNA, 12 bp, synthetic construct
  misc_feature 1..12: note = Code sequence of SKIK Tag
  source 1..12: mol_type = other DNA
tcgaagatcaag

SEQ ID NO: 111 - DNA, 18 bp, synthetic construct
  misc_feature 1..18: note = Code sequence of VKKX Tag
  source 1..18: mol_type = other DNA
gttaagaaaaccaagaca

SEQ ID NO: 112 - DNA, 18 bp, synthetic construct
  misc_feature 1..18: note = Code sequence of VKKX Tag
  source 1..18: mol_type = other DNA
gtgaagaagaccaagacc

SEQ ID NO: 113 - protein, 80 aa, synthetic construct
  REGION 1..80: note = Fusion protein
VGSLNCIVAVSQNMGIGKNGDLPWPPLRNEFRYFQRMTTTSSVEGKQNLVIMGKKTWFSIPEKNRPGGSVSGWRLFKKIS

SEQ ID NO: 114 - protein, 100 aa, synthetic construct
  REGION 1..100: note = Fusion protein
VGSLNCIVAVSQNMGIGKNGDLPWPPLRNEFRYFQRMTTTSSVEGKQNLVIMGKKTWFSIPEKNRPLKGRINLVLSRELKEPPQGAGGSVSGWRLFKKIS

SEQ ID NO: 115 - DNA, 240 bp, synthetic construct
  source 1..240: mol_type = other DNA
  misc_feature 1..240: note = Code sequence of fusion protein
gttggatccttgaactgcatcgtagctgtgagccaaaacatgggaattgggaagaacggcgatttaccctggccaccgttgcggaatgaattccgctattttcagcgtatgaccaccacaagttcggtggaagggaaacagaatctggtgatcatgggcaagaaaacgtggtttagcattccggagaagaatcgtcctggtggctctgtaagtggatggcgattattcaagaagattagc

SEQ ID NO: 116 - DNA, 297 bp, synthetic construct
  source 1..297: mol_type = other DNA
  misc_feature 1..297: note = Code sequence of fusion protein
gttggatccttgaactgcatcgtagctgtgagccaaaacatgggaattgggaagaacggcgatttaccctggccaccgttgcggaatgaattccgctattttcagcgtatgaccaccacaagttcggtggaagggaaacagaatctggtgatcggcaagaaaacgtggtttagcattccggagaagaatcgtcctctgaaaggccgtatcaacctcgttctgtcacgcgaactgaaagagcctccacaaggtgcaggtggctctgtaagtggatggcgattattcaagaagattagc

SEQ ID NO: 117 - DNA, 558 bp, synthetic construct
  source 1..558: mol_type = other DNA
  misc_feature 1..558: note = Code sequence of DHRF
gttggatccttgaactgcatcgtagctgtgagccaaaacatgggaattgggaagaacggcgatttaccctggccaccgttgcggaatgaattccgctattttcagcgtatgaccaccacaagttcggtggaagggaaacagaatctggtgatcatgggcaagaaaacgtggtttagcattccggagaagaatcgtcctctgaaaggccgtatcaacctcgttctgtcacgcgaactgaaagagcctccacaaggtgcacacttccttagccgcagtcttgatgatgccctgaaactgactgaacagcccgaattagcgaacaaagtcgatatggtctggattgtaggtggctcttccgtgtacaaagaagcgatgaatcatccgggtcatctgaaactgtttgttacgcgcattatgcaggactttgaatcggataccttctttccggaaattgacctcgagaaatacaaactgttaccggaatatccgggtgttctgtctgatgtgcaggaagagaaaggcatcaaatacaaattcgaagtctatgagaagaacgac

SEQ ID NO: 118 - DNA, 55 bp, synthetic construct
  source 1..55: mol_type = other DNA
  misc_feature 1..55: note = Forward primer for VKKTKT tag
aaggagatataccaatggttaaaaaaacaaaaacagttggatccttgaactgcat

SEQ ID NO: 119 - DNA, 49 bp, synthetic construct
  source 1..49: mol_type = other DNA
  misc_feature 1..49: note = Forward primer for SKIK tag
aaggagatataccaatgtcgaagatcaaggttggatccttgaactgcat

SEQ ID NO: 120 - DNA, 20 bp, synthetic construct
  source 1..20: mol_type = other DNA
  misc_feature 1..20: note = 1st reverse primer
ttagtcgttcttctcataga

SEQ ID NO: 121 - DNA, 21 bp, synthetic construct
  source 1..21: mol_type = other DNA
  misc_feature 1..21: note = 2nd reverse primer
aggacgattcttctccggaat

SEQ ID NO: 122 - DNA, 21 bp, synthetic construct
  source 1..21: mol_type = other DNA
  misc_feature 1..21: note = 2nd reverse primer
tgcaccttgtggaggctcttt

SEQ ID NO: 123 - DNA, 80 bp, synthetic construct
  source 1..80: mol_type = other DNA
ggattagttattcattagctaatcttcttgaataatcgccatccacttacagagccaccaggacgattcttctccggaat

SEQ ID NO: 124 - DNA, 80 bp, synthetic construct
  source 1..80: mol_type = other DNA
ggattagttattcattagctaatcttcttgaataatcgccatccacttacagagccacctgcaccttgtggaggctcttt

SEQ ID NO: 125 - protein, 24 aa, synthetic construct
EQKLISEEDLGGSVSGWRLFKKIS

SEQ ID NO: 126 - protein, 16 aa, synthetic construct
  SITE 10: note = Chloroacetyl lysine
CEPRGDNYRXGGSKKK

SEQ ID NO: 127 - DNA, 202 bp, synthetic construct
  source 1..202: mol_type = other DNA
  misc_feature 89..106: note = VKKX Tag
gaaattaatacgactcactatagggagaccacaacggtttccctctagaaataattttgtttaactttaagaaggagatatacatatggttaagaaaacaaaaacannntgtnnnnnnnnnnnnnnnnnnnnnnnntagnnnggtggctctggcggtagcaggacggggggcggcggggggtaaataaataagcttgagtat

SEQ ID NO: 128 - DNA, 199 bp, synthetic construct
  source 1..199: mol_type = other DNA
  misc_feature 89..106: note = VKKX Tag
gaaattaatacgactcactatagggagaccacaacggtttccctctagaaataattttgtttaactttaagaaggagatatacatatggttaagaaaacaaaaacannntgtnnnnnnnnnnnnnnnnnnnnnnnntagnnnggtggctctggcggtagcggcggggggcgggaggcgggaataaataagcttgagtat

SEQ ID NO: 129 - DNA, 105 bp, synthetic construct
  source 1..105: mol_type = other DNA
gaaattaatacgactcactatagggagaccacaacggtttccctctagaaataattttgtttaactttaagaaggagatatacatatggttaaaaaaacaaaaac

SEQ ID NO: 130 - DNA, 92 bp, synthetic construct
  source 1..92: mol_type = other DNA
aagaaggagatatacatatggttaaaaaaacaaaaacannntgtnnnnnnnnnnnnnnnnnnnnnnnntagnnnggcggttctggcggtagc

SEQ ID NO: 131 - DNA, 63 bp, synthetic construct
  source 1..63: mol_type = other DNA
atactcaagcttatttatttattaccccccgccgccccccgtcctgctaccgccagaaccacc

SEQ ID NO: 132 - DNA, 61 bp, synthetic construct
  source 1..61: mol_type = other DNA
atactcaagcttatttatttatcccgcctcccgccccccgtccgctaccgccagaaccacc

SEQ ID NO: 133 - DNA, 23 bp, synthetic construct
  source 1..23: mol_type = other DNA
taccccccgccgccccccgtcct

SEQ ID NO: 134 - RNA, 23 nt, synthetic construct
  source 1..23: mol_type = other RNA
  modified_base 1: mod_base = um
  modified_base 2: mod_base = OTHER; note = 2'-O-methyladenosine
  modified_base 3..8: mod_base = cm
  modified_base 9: mod_base = gm
  modified_base 10..11: mod_base = cm
  modified_base 11: mod_base = gm
  modified_base 13..18: mod_base = cm
  modified_base 19: mod_base = gm
  modified_base 20: mod_base = um
  modified_base 21..22: mod_base = cm
  modified_base 23: mod_base = um
taccccccgccgccccccgtcct

SEQ ID NO: 135 - RNA, 23 nt, synthetic construct
  source 1..23: mol_type = other RNA
  modified_base 1: mod_base = um
  modified_base 2: mod_base = OTHER; note = 2'-O-methyladenosine
  modified_base 3..8: mod_base = cm
  modified_base 9: mod_base = gm
  modified_base 10..11: mod_base = cm
  modified_base 12: mod_base = gm
  modified_base 13..18: mod_base = cm
  modified_base 19: mod_base = gm
  modified_base 20: mod_base = um
  modified_base 21..22: mod_base = cm
  modified_base 23: mod_base = um
taccccccgccgccccccgtcct

SEQ ID NO: 136 - RNA, 21 nt, synthetic construct
  source 1..21: mol_type = other RNA
  modified_base 1..3: mod_base = cm
  modified_base 4: mod_base = gm
  modified_base 5..6: mod_base = cm
  modified_base 7: mod_base = um
  modified_base 8..10: mod_base = cm
  modified_base 11: mod_base = gm
  modified_base 12..17: mod_base = cm
  modified_base 18: mod_base = gm
  modified_base 19: mod_base = um
  modified_base 20..21: mod_base = cm
cccgcctcccgccccccgtcc

SEQ ID NO: 137 - DNA, 18 bp, synthetic construct
  source 1..18: mol_type = other DNA
gctaccgccagaaccacc

SEQ ID NO: 138 - DNA, 32 bp, synthetic construct
  source 1..32: mol_type = other DNA
ggagatatacatatggttaagaaaacaaaaac

SEQ ID NO: 139 - DNA, 20 bp, synthetic construct
  source 1..20: mol_type = other DNA
ctgctaccgccagaaccacc